European Patent Specification EP 3 656 786 B1, published August 28, 2024. Title: ANTI-IL-17A ANTIBODIES AND THEIR USE IN TREATING AUTOIMMUNE AND INFLAMMATORY DISORDERS. Applicant: Novartis AG. Application PCT/IB2014/058854. The sequence listing filed with the application follows.

SEQUENCE LISTING (86 sequences)

SEQ ID NO: 1 - protein, 7 aa, Homo sapiens
GFTFSSY

SEQ ID NO: 2 - protein, 6 aa, Homo sapiens
KQDGSE

SEQ ID NO: 3 - protein, 7 aa, Homo sapiens
DRGSLYY

SEQ ID NO: 4 - protein, 7 aa, Homo sapiens
SQGIISA

SEQ ID NO: 5 - protein, 3 aa, Homo sapiens
DAS

SEQ ID NO: 6 - protein, 6 aa, Homo sapiens
FNSYPL

SEQ ID NO: 7 - protein, 5 aa, Homo sapiens
SYWMS

SEQ ID NO: 8 - protein, 17 aa, Homo sapiens
NIKQDGSEKYYVDSVKG

SEQ ID NO: 9 - protein, 11 aa, Homo sapiens
RPSQGIISALA

SEQ ID NO: 10 - protein, 7 aa, Homo sapiens
DASSLEN

SEQ ID NO: 11 - protein, 9 aa, Homo sapiens
QQFNSYPLT

SEQ ID NO: 12 - protein, 116 aa, Homo sapiens
EVQLVESGGDLVQPGGSLRLSCAASGFTFSSYWMSWVRQAPGKGLEWVANIKQDGSEKYYVDSVKGRFTISRDNAKNSLYLQMNSLRAEDTAVYYCARDRGSLYYWGQGTLVTVSS

SEQ ID NO: 13 - protein, 107 aa, Homo sapiens
AIQLTQSPSSLSASVGDRVTITCRPSQGIISALAWYQQKPGKAPKLLIYDASSLENGVPSRFSGSGSGTDFTLTISSLQPEDFATYYCQQFNSYPLTFGGGTKVEIK

SEQ ID NO: 14 - protein, 446 aa, Homo sapiens
EVQLVESGGDLVQPGGSLRLSCAASGFTFSSYWMSWVRQAPGKGLEWVANIKQDGSEKYYVDSVKGRFTISRDNAKNSLYLQMNSLRAEDTAVYYCARDRGSLYYWGQGTLVTVSSASTKGPSVFPLAPSSKSTSGGTAALGCLVKDYFPEPVTVSWNSGALTSGVHTFPAVLQSSGLYSLSSVVTVPSSSLGTQTYICNVNHKPSNTKVDKRVEPKSCDKTHTCPPCPAPELLGGPSVFLFPPKPKDTLMISRTPEVTCVVVDVSHEDPEVKFNWYVDGVEVHNAKTKPREEQYNSTYRVVSVLTVLHQDWLNGKEYKCKVSNKALPAPIEKTISKAKGQPREPQVYTLPPSREEMTKNQVSLTCLVKGFYPSDIAVEWESNGQPENNYKTTPPVLDSDGSFFLYSKLTVDKSRWQQGNVFSCSVMHEALHNHYTQKSLSLSPGK

SEQ ID NO: 15 - protein, 214 aa, Homo sapiens
AIQLTQSPSSLSASVGDRVTITCRPSQGIISALAWYQQKPGKAPKLLIYDASSLENGVPSRFSGSGSGTDFTLTISSLQPEDFATYYCQQFNSYPLTFGGGTKVEIKRTVAAPSVFIFPPSDEQLKSGTASVVCLLNNFYPREAKVQWKVDNALQSGNSQESVTEQDSKDSTYSLSSTLTLSKADYEKHKVYACEVTHQGLSSPVTKSFNRGEC

SEQ ID NO: 16 - DNA, 348 bp, Homo sapiens
gaggtgcagctggtcgagtctggcggcgacctggtgcagcctggcggcagcctgagactgagctgcgccgccagcggcttcaccttcagcagctactggatgtcctgggtccgccaggcccctggcaaaggcctcgaatgggtggccaacatcaagcaggacggcagcgagaagtactacgtggacagcgtgaagggccggttcaccatcagccgggacaacgccaagaacagcctgtacctgcagatgaacagcctgcgggccgaggacaccgccgtgtactactgcgccagggaccggggcagcctgtactattggggccagggcaccctggtcaccgtgtccagc

SEQ ID NO: 17 - DNA, 321 bp, Homo sapiens
gccatccagttgacccagtctccatcctccctgtctgcatctgtgggagacagagtcaccatcacttgccggccaagtcagggcattatcagtgctttagcctggtatcagcagaaaccagggaaagctcctaagctcctgatctatgatgcctccagtttggaaaatggggtcccatcaaggttcagcggcagtggatctgggacagatttcactctcaccatcagcagcctgcagcctgaagattttgcaacttattactgtcaacagtttaatagttaccctctcactttcggcggagggaccaaggtggagatcaaa

SEQ ID NO: 18 - DNA, 1338 bp, Homo sapiens
gaggtgcagctggtcgagtctggcggcgacctggtgcagcctggcggcagcctgagactgagctgcgccgccagcggcttcaccttcagcagctactggatgtcctgggtccgccaggcccctggcaaaggcctcgaatgggtggccaacatcaagcaggacggcagcgagaagtactacgtggacagcgtgaagggccggttcaccatcagccgggacaacgccaagaacagcctgtacctgcagatgaacagcctgcgggccgaggacaccgccgtgtactactgcgccagggaccggggcagcctgtactattggggccagggcaccctggtcaccgtgtccagcgctagcaccaagggccccagcgtgttccccctggcccccagcagcaagagcaccagcggcggcacagccgccctgggctgcctggtgaaggactacttccccgagcccgtgaccgtgtcctggaacagcggagccctgacctccggcgtgcacaccttccccgccgtgctgcagagcagcggcctgtacagcctgtccagcgtggtgacagtgcccagcagcagcctgggcacccagacctacatctgcaacgtgaaccacaagcccagcaacaccaaggtggacaagagagtggagcccaagagctgcgacaagacccacacctgccccccctgcccagccccagagctgctgggcggaccctccgtgttcctgttcccccccaagcccaaggacaccctgatgatcagcaggacccccgaggtgacctgcgtggtggtggacgtgagccacgaggacccagaggtgaagttcaactggtacgtggacggcgtggaggtgcacaacgccaagaccaagcccagagaggagcagtacaacagcacctacagggtggtgtccgtgctgaccgtgctgcaccaggactggctgaacggcaaggaatacaagtgcaaggtctccaacaaggccctgccagcccccatcgaaaagaccatcagcaaggccaagggccagccacgggagccccaggtgtacaccctgcccccctcccgggaggagatgaccaagaaccaggtgtccctgacctgtctggtgaagggcttctaccccagcgacatcgccgtggagtgggagagcaacggccagcccgagaacaactacaagaccacccccccagtgctggacagcgacggcagcttcttcctgtacagcaagctgaccgtggacaagtccaggtggcagcagggcaacgtgttcagctgcagcgtgatgcacgaggccctgcacaaccactacacccagaagagcctgagcctgtcccccggcaag

SEQ ID NO: 19 - DNA, 642 bp, Homo sapiens
gccatccagttgacccagtctccatcctccctgtctgcatctgtgggagacagagtcaccatcacttgccggccaagtcagggcattatcagtgctttagcctggtatcagcagaaaccagggaaagctcctaagctcctgatctatgatgcctccagtttggaaaatggggtcccatcaaggttcagcggcagtggatctgggacagatttcactctcaccatcagcagcctgcagcctgaagattttgcaacttattactgtcaacagtttaatagttaccctctcactttcggcggagggaccaaggtggagatcaaacgtacggtggccgctcccagcgtgttcatcttcccccccagcgacgagcagctgaagagcggcaccgccagcgtggtgtgcctgctgaacaacttctacccccgggaggccaaggtgcagtggaaggtggacaacgccctgcagagcggcaacagccaggagagcgtcaccgagcaggacagcaaggactccacctacagcctgagcagcaccctgaccctgagcaaggccgactacgagaagcataaggtgtacgcctgcgaggtgacccaccagggcctgtccagccccgtgaccaagagcttcaacaggggcgagtgc

SEQ ID NO: 20 - protein, 7 aa, Homo sapiens
SQVIISA

SEQ ID NO: 21 - protein, 6 aa, Homo sapiens
FDSYPL

SEQ ID NO: 22 - protein, 11 aa, Homo sapiens
RPSQVIISALA

SEQ ID NO: 23 - protein, 7 aa, Homo sapiens
DASSLEQ

SEQ ID NO: 24 - protein, 9 aa, Homo sapiens
QQFDSYPLT

SEQ ID NO: 25 - protein, 107 aa, Homo sapiens
AIQLTQSPSSLSASVGDRVTITCRPSQVIISALAWYQQKPGKAPKLLIYDASSLEQGVPSRFSGSVSGTDFTLTISSLQPEDFATYYCQQFDSYPLTFGGGTKVEIK

SEQ ID NO: 26 - protein, 214 aa, Homo sapiens
AIQLTQSPSSLSASVGDRVTITCRPSQVIISALAWYQQKPGKAPKLLIYDASSLEQGVPSRFSGSVSGTDFTLTISSLQPEDFATYYCQQFDSYPLTFGGGTKVEIKRTVAAPSVFIFPPSDEQLKSGTASVVCLLNNFYPREAKVQWKVDNALQSGNSQESVTEQDSKDSTYSLSSTLTLSKADYEKHKVYACEVTHQGLSSPVTKSFNRGEC

SEQ ID NO: 27 - DNA, 321 bp, Homo sapiens
gccatccagctgacccagagccccagcagcctgagcgccagcgtgggcgacagagtgaccatcacctgtcggcccagccaggtcatcatcagcgccctggcctggtatcagcagaagcctggcaaggcccccaagctgctgatctacgacgccagctccctggaacagggcgtgcccagccggttcagcggcagcgtgtccggcaccgacttcaccctgaccatcagctccctgcagcccgaggacttcgccacctactactgccagcagttcgacagctaccccctgaccttcggcggaggcaccaaggtggaaatcaag

SEQ ID NO: 28 - DNA, 642 bp, Homo sapiens
gccatccagctgacccagagccccagcagcctgagcgccagcgtgggcgacagagtgaccatcacctgtcggcccagccaggtcatcatcagcgccctggcctggtatcagcagaagcctggcaaggcccccaagctgctgatctacgacgccagctccctggaacagggcgtgcccagccggttcagcggcagcgtgtccggcaccgacttcaccctgaccatcagctccctgcagcccgaggacttcgccacctactactgccagcagttcgacagctaccccctgaccttcggcggaggcaccaaggtggaaatcaagcgtacggtggccgctcccagcgtgttcatcttcccccccagcgacgagcagctgaagagcggcaccgccagcgtggtgtgcctgctgaacaacttctacccccgggaggccaaggtgcagtggaaggtggacaacgccctgcagagcggcaacagccaggagagcgtcaccgagcaggacagcaaggactccacctacagcctgagcagcaccctgaccctgagcaaggccgactacgagaagcataaggtgtacgcctgcgaggtgacccaccagggcctgtccagccccgtgaccaagagcttcaacaggggcgagtgc

SEQ ID NO: 29 - DNA, 348 bp, Homo sapiens
gaggtgcagctggtggaatcaggaggcgacctggtgcagcctggcggctcactgagactgagctgcgccgctagtggcttcacctttagtagctactggatgagctgggtgcgacaggcccctggcaagggactggagtgggtggccaatattaagcaggacggctcagagaagtactacgtggactcagtgaagggccggttcactattagccgggataacgctaagaatagcctgtacctgcagatgaatagcctgagagccgaggacaccgccgtgtactactgcgctagagatagaggctcactgtactactggggccagggcaccctggtgacagtgtcttct

SEQ ID NO: 30 - DNA, 321 bp, Homo sapiens
gctattcagctgactcagtcacctagtagcctgagcgctagtgtgggcgatagagtgactatcacctgtagacctagtcaggtgatcattagcgccctggcctggtatcagcagaagcccggcaaggcccctaagctgctgatctacgacgctagtagtctggaacagggcgtgccctctaggtttagcggctcagtgtcaggcaccgacttcaccctgactattagtagcctgcagcccgaggacttcgctacctactactgtcagcagttcgatagctaccccctgaccttcggcggaggcactaaggtggaaatcaag

SEQ ID NO: 31 - DNA, 1338 bp, Homo sapiens
gaggtgcagctggtggaatcaggaggcgacctggtgcagcctggcggctcactgagactgagctgcgccgctagtggcttcacctttagtagctactggatgagctgggtgcgacaggcccctggcaagggactggagtgggtggccaatattaagcaggacggctcagagaagtactacgtggactcagtgaagggccggttcactattagccgggataacgctaagaatagcctgtacctgcagatgaatagcctgagagccgaggacaccgccgtgtactactgcgctagagatagaggctcactgtactactggggccagggcaccctggtgacagtgtcttctgctagcaccaagggcccaagtgtctttcccctggcccccagcagcaagtccacaagcggaggcactgcagctctgggttgtctggtgaaggactacttccccgagcccgtgacagtgtcctggaacagcggagccctgacctccggcgtgcacaccttccccgccgtgctgcagagcagcggcctgtacagcctgagcagcgtcgtgactgtgcctagttccagcctgggcacccagacctatatctgcaacgtgaaccacaagcccagcaacaccaaggtggacaagagagtggagcccaagagctgcgacaagacccacacctgccccccctgcccagctccagaactgctgggaggacccagcgtgttcctgttcccccccaagcccaaggacaccctgatgatcagcaggacccccgaggtgacctgcgtggtggtggacgtgtcccacgaggacccagaggtgaagttcaactggtacgtggacggggtggaggtgcacaacgccaagaccaagcccagagaggagcagtacaacagcacctacagggtggtgtccgtcctgacagtgctgcaccaggattggctgaacggcaaagaatacaagtgcaaagtctccaacaaggccctgccagccccaatcgaaaagacaatcagcaaggccaagggccagccacgggagccccaggtgtacaccctgccccccagccgggaggagatgaccaagaaccaggtgtccctgacctgtctggtgaagggcttctaccccagcgatatcgccgtggagtgggagagcaacggccagcccgagaacaactacaagaccacccccccagtgctggacagcgacggcagcttcttcctgtacagcaagctgaccgtggacaagtccaggtggcagcagggcaacgtgttcagctgcagcgtgatgcacgaggccctgcacaaccactacacccagaagtccctgagcctgagccccggcaag

SEQ ID NO: 32 - DNA, 642 bp, Homo sapiens
gctattcagctgactcagtcacctagtagcctgagcgctagtgtgggcgatagagtgactatcacctgtagacctagtcaggtgatcattagcgccctggcctggtatcagcagaagcccggcaaggcccctaagctgctgatctacgacgctagtagtctggaacagggcgtgccctctaggtttagcggctcagtgtcaggcaccgacttcaccctgactattagtagcctgcagcccgaggacttcgctacctactactgtcagcagttcgatagctaccccctgaccttcggcggaggcactaaggtggaaatcaagcgtacggtggccgctcccagcgtgttcatcttcccccccagcgacgagcagctgaagagcggcaccgccagcgtggtgtgcctgctgaacaacttctacccccgggaggccaaggtgcagtggaaggtggacaacgccctgcagagcggcaacagccaggagagcgtcaccgagcaggacagcaaggactccacctacagcctgagcagcaccctgaccctgagcaaggccgactacgagaagcataaggtgtacgcctgcgaggtgacccaccagggcctgtccagccccgtgaccaagagcttcaacaggggcgagtgc

SEQ ID NO: 33 - protein, 7 aa, Homo sapiens
SQGIYWE

SEQ ID NO: 34 - protein, 11 aa, Homo sapiens
RPSQGIYWELA

SEQ ID NO: 35 - protein, 107 aa, Homo sapiens
AIQLTQSPSSLSASVGDRVTITCRPSQGIYWELAWYQQKPGKAPKLLIYDASSLEQGVPSRFSGSGSGTDFTLTISSLQPEDFATYYCQQFNSYPLTFGGGTKVEIK

SEQ ID NO: 36 - protein, 214 aa, Homo sapiens
AIQLTQSPSSLSASVGDRVTITCRPSQGIYWELAWYQQKPGKAPKLLIYDASSLEQGVPSRFSGSGSGTDFTLTISSLQPEDFATYYCQQFNSYPLTFGGGTKVEIKRTVAAPSVFIFPPSDEQLKSGTASVVCLLNNFYPREAKVQWKVDNALQSGNSQESVTEQDSKDSTYSLSSTLTLSKADYEKHKVYACEVTHQGLSSPVTKSFNRGEC

SEQ ID NO: 37 - DNA, 321 bp, Homo sapiens
gccatccagctgacccagagccccagcagcctgagcgccagcgtgggcgacagagtgaccatcacctgtcggcccagccagggcatctactgggagctggcctggtatcagcagaagcctggcaaggcccccaagctgctgatctacgacgccagctccctggaacagggcgtgcccagccggttcagcggcagcggatccggcaccgacttcaccctgaccatcagctccctgcagcccgaggacttcgccacctactactgccagcagttcaacagctaccccctgaccttcggcggaggcaccaaggtggaaatcaag

SEQ ID NO: 38 - DNA, 642 bp, Homo sapiens
gccatccagctgacccagagccccagcagcctgagcgccagcgtgggcgacagagtgaccatcacctgtcggcccagccagggcatctactgggagctggcctggtatcagcagaagcctggcaaggcccccaagctgctgatctacgacgccagctccctggaacagggcgtgcccagccggttcagcggcagcggatccggcaccgacttcaccctgaccatcagctccctgcagcccgaggacttcgccacctactactgccagcagttcaacagctaccccctgaccttcggcggaggcaccaaggtggaaatcaagcgtacggtggccgctcccagcgtgttcatcttcccccccagcgacgagcagctgaagagcggcaccgccagcgtggtgtgcctgctgaacaacttctacccccgggaggccaaggtgcagtggaaggtggacaacgccctgcagagcggcaacagccaggagagcgtcaccgagcaggacagcaaggactccacctacagcctgagcagcaccctgaccctgagcaaggccgactacgagaagcataaggtgtacgcctgcgaggtgacccaccagggcctgtccagccccgtgaccaagagcttcaacaggggcgagtgc

SEQ ID NO: 39 - DNA, 321 bp, Homo sapiens
gctattcagctgactcagtcacctagtagcctgagcgctagtgtgggcgatagagtgactatcacctgtagacctagccagggaatctactgggagctggcctggtatcagcagaagcccggcaaggcccctaagctgctgatctacgacgctagtagtctggaacagggcgtgccctctaggtttagcggctcaggctcaggcaccgacttcaccctgactattagtagcctgcagcccgaggacttcgctacctactactgtcagcagtttaactcctaccccctgaccttcggcggaggcactaaggtggaaatcaag

SEQ ID NO: 40 - DNA, 642 bp, Homo sapiens
gctattcagctgactcagtcacctagtagcctgagcgctagtgtgggcgatagagtgactatcacctgtagacctagccagggaatctactgggagctggcctggtatcagcagaagcccggcaaggcccctaagctgctgatctacgacgctagtagtctggaacagggcgtgccctctaggtttagcggctcaggctcaggcaccgacttcaccctgactattagtagcctgcagcccgaggacttcgctacctactactgtcagcagtttaactcctaccccctgaccttcggcggaggcactaaggtggaaatcaagcgtacggtggccgctcccagcgtgttcatcttcccccccagcgacgagcagctgaagagcggcaccgccagcgtggtgtgcctgctgaacaacttctacccccgggaggccaaggtgcagtggaaggtggacaacgccctgcagagcggcaacagccaggagagcgtcaccgagcaggacagcaaggactccacctacagcctgagcagcaccctgaccctgagcaaggccgactacgagaagcataaggtgtacgcctgcgaggtgacccaccagggcctgtccagccccgtgaccaagagcttcaacaggggcgagtgc

SEQ ID NO: 41 - protein, 7 aa, Homo sapiens
SQGINWE

SEQ ID NO: 42 - protein, 11 aa, Homo sapiens
RPSQGINWELA

SEQ ID NO: 43 - protein, 107 aa, Homo sapiens
AIQLTQSPSSLSASVGDRVTITCRPSQGINWELAWYQQKPGKAPKLLIYDASSLEQGVPSRFSGSGSGTDFTLTISSLQPEDFATYYCQQFNSYPLTFGGGTKVEIK

SEQ ID NO: 44 - protein, 214 aa, Homo sapiens
AIQLTQSPSSLSASVGDRVTITCRPSQGINWELAWYQQKPGKAPKLLIYDASSLEQGVPSRFSGSGSGTDFTLTISSLQPEDFATYYCQQFNSYPLTFGGGTKVEIKRTVAAPSVFIFPPSDEQLKSGTASVVCLLNNFYPREAKVQWKVDNALQSGNSQESVTEQDSKDSTYSLSSTLTLSKADYEKHKVYACEVTHQGLSSPVTKSFNRGEC

SEQ ID NO: 45 - DNA, 321 bp, Homo sapiens
gccatccagctgacccagagccccagcagcctgagcgccagcgtgggcgacagagtgaccatcacctgtcggcccagccagggcatcaactgggagctggcctggtatcagcagaagcctggcaaggcccccaagctgctgatctacgacgccagctccctggaacagggcgtgcccagccggttcagcggcagcggatccggcaccgacttcaccctgaccatcagctccctgcagcccgaggacttcgccacctactactgccagcagttcaacagctaccccctgaccttcggcggaggcaccaaggtggaaatcaag

SEQ ID NO: 46 - DNA, 642 bp, Homo sapiens
gccatccagctgacccagagccccagcagcctgagcgccagcgtgggcgacagagtgaccatcacctgtcggcccagccagggcatcaactgggagctggcctggtatcagcagaagcctggcaaggcccccaagctgctgatctacgacgccagctccctggaacagggcgtgcccagccggttcagcggcagcggatccggcaccgacttcaccctgaccatcagctccctgcagcccgaggacttcgccacctactactgccagcagttcaacagctaccccctgaccttcggcggaggcaccaaggtggaaatcaagcgtacggtggccgctcccagcgtgttcatcttcccccccagcgacgagcagctgaagagcggcaccgccagcgtggtgtgcctgctgaacaacttctacccccgggaggccaaggtgcagtggaaggtggacaacgccctgcagagcggcaacagccaggagagcgtcaccgagcaggacagcaaggactccacctacagcctgagcagcaccctgaccctgagcaaggccgactacgagaagcataaggtgtacgcctgcgaggtgacccaccagggcctgtccagccccgtgaccaagagcttcaacaggggcgagtgc

SEQ ID NO: 47 - DNA, 321 bp, Homo sapiens
gctattcagctgactcagtcacctagtagcctgagcgctagtgtgggcgatagagtgactatcacctgtagacctagtcaggggattaactgggagctggcctggtatcagcagaagcccggcaaggcccctaagctgctgatctacgacgctagtagtctggaacagggcgtgccctctaggtttagcggctcaggctcaggcaccgacttcaccctgactattagtagcctgcagcccgaggacttcgctacctactactgtcagcagtttaactcctaccccctgaccttcggcggaggcactaaggtggaaatcaag

SEQ ID NO: 48 - DNA, 642 bp, Homo sapiens
gctattcagctgactcagtcacctagtagcctgagcgctagtgtgggcgatagagtgactatcacctgtagacctagtcaggggattaactgggagctggcctggtatcagcagaagcccggcaaggcccctaagctgctgatctacgacgctagtagtctggaacagggcgtgccctctaggtttagcggctcaggctcaggcaccgacttcaccctgactattagtagcctgcagcccgaggacttcgctacctactactgtcagcagtttaactcctaccccctgaccttcggcggaggcactaaggtggaaatcaagcgtacggtggccgctcccagcgtgttcatcttcccccccagcgacgagcagctgaagagcggcaccgccagcgtggtgtgcctgctgaacaacttctacccccgggaggccaaggtgcagtggaaggtggacaacgccctgcagagcggcaacagccaggagagcgtcaccgagcaggacagcaaggactccacctacagcctgagcagcaccctgaccctgagcaaggccgactacgagaagcataaggtgtacgcctgcgaggtgacccaccagggcctgtccagccccgtgaccaagagcttcaacaggggcgagtgc

SEQ ID NO: 49 - DNA, 348 bp, Homo sapiens
gaggtgcagctggtggaatctggcggcgacctggtgcagcctggcggctctctgagactgtcttgcgccgcctccggcttcaccttctccagctactggatgtcctgggtgcgacaggcccctggcaagggactggaatgggtggccaacatcaagcaggacggctccgagaagtactacgtggactccgtgaagggccggttcaccatctcccgggacaacgccaagaactccctgtacctgcagatgaactccctgcgggccgaggacaccgccgtgtactactgcgccagggaccggggctccctgtactattggggccagggcaccctggtgacagtgtcctcc

SEQ ID NO: 50 - DNA, 321 bp, Homo sapiens
gccatccagctgacccagtccccctccagcctgtctgcctccgtgggcgacagagtgaccatcacctgtcggccctcccagggcatcaactgggaactggcctggtatcagcagaagcccggcaaggcccccaagctgctgatctacgacgccagctccctggaacagggcgtgccctccagattctccggctctggctccggcaccgacttcaccctgaccatctccagcctgcagcccgaggacttcgccacctactactgccagcagttcaactcctaccccctgaccttcggcggaggcaccaaggtggaaatcaag

SEQ ID NO: 51 - DNA, 1338 bp, Homo sapiens
gaggtgcagctggtggaatctggcggcgacctggtgcagcctggcggctctctgagactgtcttgcgccgcctccggcttcaccttctccagctactggatgtcctgggtgcgacaggcccctggcaagggactggaatgggtggccaacatcaagcaggacggctccgagaagtactacgtggactccgtgaagggccggttcaccatctcccgggacaacgccaagaactccctgtacctgcagatgaactccctgcgggccgaggacaccgccgtgtactactgcgccagggaccggggctccctgtactattggggccagggcaccctggtgacagtgtcctccgcctccaccaagggcccaagcgtgttccccctggcccccagcagcaagagcaccagcggcggcacagccgccctgggctgcctggtgaaggactacttccccgagcccgtgaccgtgtcctggaacagcggagccctgacctccggcgtgcacaccttccccgccgtgctgcagagcagcggcctgtacagcctgagcagcgtggtgaccgtgcccagcagcagcctgggcacccagacctacatctgtaacgtgaaccacaagcccagcaacaccaaggtggacaagagagtggagcccaagagctgtgacaagacccacacctgccccccctgcccagcccccgagctgctgggcggacccagcgtgttcctgttcccccccaagcccaaggacaccctgatgatcagcagaacccccgaggtgacctgtgtggtggtggacgtgtcccacgaggacccagaggtgaagttcaactggtacgtggacggcgtggaggtgcacaacgccaagaccaagcccagagaggagcagtacaacagcacctacagggtggtgtccgtgctgaccgtgctgcaccaggactggctgaacggcaaggagtacaagtgtaaggtgtccaacaaggccctgccagccccaatcgaaaagaccatcagcaaggccaagggccagccaagagagccccaggtgtacaccctgccacccagcagggaggagatgaccaagaaccaggtgtccctgacctgtctggtgaagggcttctacccaagcgacatcgccgtggagtgggagagcaacggccagcccgagaacaactacaagaccacccccccagtgctggacagcgacggcagcttcttcctgtacagcaagctgaccgtggacaagagcagatggcagcagggcaacgtgttcagctgctccgtgatgcacgaggccctgcacaaccactacacccagaagagcctgagcctgtccccaggcaag

SEQ ID NO: 52 - DNA, 642 bp, Homo sapiens
gccatccagctgacccagtccccctccagcctgtctgcctccgtgggcgacagagtgaccatcacctgtcggccctcccagggcatcaactgggaactggcctggtatcagcagaagcccggcaaggcccccaagctgctgatctacgacgccagctccctggaacagggcgtgccctccagattctccggctctggctccggcaccgacttcaccctgaccatctccagcctgcagcccgaggacttcgccacctactactgccagcagttcaactcctaccccctgaccttcggcggaggcaccaaggtggaaatcaagcgtacggtggccgctcccagcgtgttcatcttccccccaagcgacgagcagctgaagagcggcaccgccagcgtggtgtgtctgctgaacaacttctaccccagggaggccaaggtgcagtggaaggtggacaacgccctgcagagcggcaacagccaggagagcgtcaccgagcaggacagcaaggactccacctacagcctgagcagcaccctgaccctgagcaaggccgactacgagaagcacaaggtgtacgcctgtgaggtgacccaccagggcctgtccagccccgtgaccaagagcttcaacaggggcgagtgc

SEQ ID NO: 53 - protein, 107 aa, Homo sapiens
AIQLTQSPSSLSASVGDRVTITCRPSQGINWELAWYQQKPGKAPKLLIYDASSLENGVPSRFSGSGSGTDFTLTISSLQPEDFATYYCQQFNSYPLTFGGGTKVEIK

SEQ ID NO: 54 - protein, 214 aa, Homo sapiens
AIQLTQSPSSLSASVGDRVTITCRPSQGINWELAWYQQKPGKAPKLLIYDASSLENGVPSRFSGSGSGTDFTLTISSLQPEDFATYYCQQFNSYPLTFGGGTKVEIKRTVAAPSVFIFPPSDEQLKSGTASVVCLLNNFYPREAKVQWKVDNALQSGNSQESVTEQDSKDSTYSLSSTLTLSKADYEKHKVYACEVTHQGLSSPVTKSFNRGEC

SEQ ID NO: 55 - DNA, 321 bp, Homo sapiens
gccatccagctgacccagagccccagcagcctgagcgccagcgtgggcgacagagtgaccatcacctgtcggcccagccagggcatcaactgggagctggcctggtatcagcagaagcctggcaaggcccccaagctgctgatctacgacgccagctccctggaaaacggcgtgcccagccggttcagcggcagcggatccggcaccgacttcaccctgaccatcagctccctgcagcccgaggacttcgccacctactactgccagcagttcaacagctaccccctgaccttcggcggaggcaccaaggtggaaatcaag

SEQ ID NO: 56 - DNA, 642 bp, Homo sapiens
gccatccagctgacccagagccccagcagcctgagcgccagcgtgggcgacagagtgaccatcacctgtcggcccagccagggcatcaactgggagctggcctggtatcagcagaagcctggcaaggcccccaagctgctgatctacgacgccagctccctggaaaacggcgtgcccagccggttcagcggcagcggatccggcaccgacttcaccctgaccatcagctccctgcagcccgaggacttcgccacctactactgccagcagttcaacagctaccccctgaccttcggcggaggcaccaaggtggaaatcaagcgtacggtggccgctcccagcgtgttcatcttcccccccagcgacgagcagctgaagagcggcaccgccagcgtggtgtgcctgctgaacaacttctacccccgggaggccaaggtgcagtggaaggtggacaacgccctgcagagcggcaacagccaggagagcgtcaccgagcaggacagcaaggactccacctacagcctgagcagcaccctgaccctgagcaaggccgactacgagaagcataaggtgtacgcctgcgaggtgacccaccagggcctgtccagccccgtgaccaagagcttcaacaggggcgagtgc

SEQ ID NO: 57 - DNA, 321 bp, Homo sapiens
gctattcagctgactcagtcacctagtagcctgagcgctagtgtgggcgatagagtgactatcacctgtagacctagtcaggggattaactgggagctggcctggtatcagcagaagcccggcaaggcccctaagctgctgatctacgacgctagtagtctggaaaacggcgtgccctctaggtttagcggctcaggctcaggcaccgacttcaccctgactattagtagcctgcagcccgaggacttcgctacctactactgtcagcagtttaactcctaccccctgaccttcggcggaggcactaaggtggaaatcaag

SEQ ID NO: 58 - DNA, 642 bp, Homo sapiens
gctattcagctgactcagtcacctagtagcctgagcgctagtgtgggcgatagagtgactatcacctgtagacctagtcaggggattaactgggagctggcctggtatcagcagaagcccggcaaggcccctaagctgctgatctacgacgctagtagtctggaaaacggcgtgccctctaggtttagcggctcaggctcaggcaccgacttcaccctgactattagtagcctgcagcccgaggacttcgctacctactactgtcagcagtttaactcctaccccctgaccttcggcggaggcactaaggtggaaatcaagcgtacggtggccgctcccagcgtgttcatcttcccccccagcgacgagcagctgaagagcggcaccgccagcgtggtgtgcctgctgaacaacttctacccccgggaggccaaggtgcagtggaaggtggacaacgccctgcagagcggcaacagccaggagagcgtcaccgagcaggacagcaaggactccacctacagcctgagcagcaccctgaccctgagcaaggccgactacgagaagcataaggtgtacgcctgcgaggtgacccaccagggcctgtccagccccgtgaccaagagcttcaacaggggcgagtgc

SEQ ID NO: 59 - protein, 19 aa, Artificial Sequence
  Heavy chain leader sequence
MEFGLSWVFLVAILEGVHC

SEQ ID NO: 60 - protein, 22 aa, Artificial sequence
  Light chain leader sequence
MDMRVPAQLLGLLLLWLPGARC

SEQ ID NO: 61 - DNA, 57 bp, Artificial sequence
  Coding sequence for heavy chain leader sequence
atggaattcggcctgagctgggtgttcctggtcgcgattctggaaggcgtgcactgc

SEQ ID NO: 62 - DNA, 66 bp, Artificial sequence
  Coding sequence for light chain leader sequence
atggacatgagggtccccgctcagctcctggggcttctgctgctctggctcccaggcgccagatgt

SEQ ID NO: 63 - protein, 19 aa, Artificial sequence
  Alternative heavy chain leader sequence
MAWVWTLPFLMAAAQSVQA

SEQ ID NO: 64 - protein, 20 aa, Artificial sequence
  Alternative light chain leader sequence
MSVLTQVLALLLLWLTGTRC

SEQ ID NO: 65 - DNA, 57 bp, Artificial sequence
  Coding sequence for alternative heavy chain leader sequence
atggcctgggtgtggaccctgcccttcctgatggccgctgctcagtcagtgcaggcc

SEQ ID NO: 66 - DNA, 60 bp, Artificial sequence
  Coding sequence for alternative light chain leader sequence
atgagcgtgctgactcaggtgctggccctgctgctgctgtggctgaccggcacccgctgc

SEQ ID NO: 67 - protein, 19 aa, Artificial sequence
  Second alternative heavy chain leader sequence
MEWSWVFLFFLSVTTGVHS

SEQ ID NO: 68 - protein, 20 aa, Artificial sequence
  Second alternative light chain leader sequence
MSVPTQVLGLLLLWLTDARC

SEQ ID NO: 69 - DNA, 57 bp, Artificial sequence
  Coding sequence for second alternative heavy chain leader sequence
atggaatggtcctgggtgttcctgttcttcctgtccgtgaccacaggcgtgcactcc

SEQ ID NO: 70 - DNA, 60 bp, Artificial sequence
  Coding sequence for second alternative light chain leader sequence
atgtccgtgcccacacaggtgctgggcctgctgctgctgtggctgaccgacgccagatgc

SEQ ID NO: 71 - protein, 7 aa, Homo sapiens
  Xaa (3)..(3): Variable
  Xaa (5)..(7): Variable
SQXIXXX

SEQ ID NO: 72 - protein, 6 aa, Homo sapiens
  Xaa (2)..(2): Variable
FXSYPL

SEQ ID NO: 73 - protein, 11 aa, Homo sapiens
  Xaa (5)..(5): Variable
  Xaa (7)..(9): Variable
RPSQXIXXXLA

SEQ ID NO: 74 - protein, 7 aa, Homo sapiens
  Xaa (7)..(7): Variable
DASSLEX

SEQ ID NO: 75 - protein, 9 aa, Homo sapiens
  Xaa (4)..(4): Variable
QQFXSYPLT

SEQ ID NO: 76 - protein, 136 aa, Homo sapiens
GITIPRNPGCPNSEDKNFPRTVMVNLNIHNRNTNTNPKRSSDYYNRSTSPWNLHRNEDPERYPSVIWEAKCRHLGCINADGNVDYHMNSVPIQQEILVLRREPPHCPNSFRLEKILVSVGCTCVTPIVHHVAEFRH

SEQ ID NO: 77 - protein, 134 aa, Homo sapiens
MRKIPKVGHTFFQKPESCPPVPGGSMKLDIGIINENQRVSMSRNIESRSTSPWNYTVTWDPNRYPSEVVQAQCRNLGCINAQGKEDISMNSVPIQQETLVVRRKHQGCSVSFQLEKVLVTVGCTCVTPVIHHVQ

SEQ ID NO: 78 - protein, 138 aa, Homo sapiens
GPIVKAGITIPRNPGCPNSEDKNFPRTVMVNLNIHNRNTNTNPKRSSDYYNRSTSPWNLHRNEDPERYPSVIWEAKCRHLGCINADGNVDYHMNSVPIQQEILVLRREPPHCPNSFRLEKILVSVGCTCVTPIVHHVA

SEQ ID NO: 79 - protein, 132 aa, Macaca fascicularis
GIAIPRNSGCPNSEDKNFPRTVMVNLNIHNRNTSTNPKRSSDYYNRSTSPWNLHRNEDPERYPSVIWEAKCRHLGCVKADGNVDYHMNSVPIQQEILVLRREPRHCPNSFRLEKILVSVGCTCVTPIVHHVA

SEQ ID NO: 80 - protein, 134 aa, Macaca fascicularis
MRKIPKVGHTFFQKPESCPPVPEGSMKLDTGIINENQRVSMSRNIESRSTSPWNYTVTWDPNRYPSEVVQAQCKHLGCINAQGKEDISMNSVPIQQETLVLRRKHQGCSVSFQLEKVLVTVGCTCVTPVVHHVQ

SEQ ID NO: 81 - protein, 132 aa, Macaca mulatta
GIAIPRNSGCPNSEDKNFPRTVMVNLNIHNRNTSTSPKRSSDYYNRSTSPWNLHRNEDPERYPSVIWEAKCRHLGCVKADGNVDYHMNSVPIQQEILVLRREPRHCPNSFRLEKILVSVGCTCVTPIVHHVA

SEQ ID NO: 82 - protein, 127 aa, Callithrix jacchus
SPQNPGCPNAEDKNFPRTVMVNLNIRNRNTNSKRASDYYNRSSSPWNLHRNEDPERYPSVIWEAKCRHLGCVDADGNVDYHMNSVPIQQEILVLRREPRHCTNSFRLEKMLVSVGCTCVTPIVHHVA

SEQ ID NO: 83 - protein, 134 aa, Mus musculus
MAAIIPQSSACPNTEAKDFLQNVKVNLKVFNSLGAKVSSRRPSDYLNRSTSPWTLHRNEDPDRYPSVIWEAQCRHQRCVNAEGKLDHHMNSVLIQQEILVLKREPESCPFTFRVEKMLVGVGCTCVASIVRQAA

SEQ ID NO: 84 - protein, 141 aa, Mus musculus
APEPEFRHRKNPKAGVPALQKAGNCPPLEDNTVRVDIRIFNQNQGISVPREFQNRSSSPWDYNITRDPHRFPSEIAEAQCRHSGCINAQGQEDSTMNSVAIQQEILVLRREPQGCSNSFRLEKMLLKVGCTCVKPIVHQAA

SEQ ID NO: 85 - protein, 134 aa, Rattus norvegicus
MAVLIPQSSVCPNAEANNFLQNVKVNLKVINSLSSKASSRRPSDYLNRSTSPWTLSRNEDPDRYPSVIWEAQCRHQRCVNAEGKLDHHMNSVLIQQEILVLKREPEKCPFTFRVEKMLVGVGCTCVSSIVRHAS

SEQ ID NO: 86 - protein, 295 aa, Homo sapiens
NCTVKNSTCLDDSWIHPRNLTPSSPKDLQIQLHFAHTQQGDLFPVAHIEWTLQTDASILYLEGAELSVLQLNTNERLCVRFEFLSKLRHHHRRWRFTFSHFVVDPDQEYEVTVHHLPKPIPDGDPNHQSKNFLVPDCEHARMKVTTPCMSSGSLWDPNITVETLEAHQLRVSFTLWNESTHYQILLTSFPHMENHSCFEHMHHIPAPRPEEFHQRSNVTLTLRNLKGCCRHQVQIQPFFSSCLNDCLRHSATVSCPEMPDTPEPIPDYMPLWEFRHDSGGGLNDIFEAQKIEWHE